European Patent Specification EP 3 399 025 B1, published May 7, 2025. Title: SOMATIC CELL REPROGRAMMING. Applicant: Wisconsin Alumni Research Foundation. The sequence listing filed with the application follows.

SEQUENCE LISTING (13 sequences)

SEQ ID NO: 1 - DNA, 480 bp, Stella
atggacccatcacagtttaatccaacctacatcccagggtctccacaaatgctcaccgaagaaaattcccgggacgattcaggggcctctcaaatctcctccgagacgttgataaagaaccttagtaacttgactatcaacgctagtagcgaatctgtttcccctctatcggaagctttactccgtcgagagtctgtaggagcagcagtcctcagggaaatcgaagatgagtggctttacagcaggagaggagtaagaacattgctgtctgtgcagagagaaaagatggcaagattgagatacatgttactcggcggagttcgtacgcatgaaagaagaccaacaaacaaggagcctaagggagttaagaaggaatcaagaccattcaaatgtccctgcagtttctgcgtgtctaatggatgggatccttctgagaatgctagaatagggaatcaagacaccaagccacttcagccataa

SEQ ID NO: 2 - DNA, 1083 bp, Oct-4
atggcgggacacctggcttcggatttcgccttctcgccccctccaggtggtggaggtgatgggccaggggggccggagccgggctgggttgatcctcggacctggctaagcttccaaggccctcctggagggccaggaatcgggccgggggttgggccaggctctgaggtgtgggggattcccccatgccccccgccgtatgagttctgtggggggatggcgtactgtgggccccaggttggagtggggctagtgccccaaggcggcttggagacctctcagcctgagggcgaagcaggagtcggggtggagagcaactccgatggggcctccccggagccctgcaccgtcacccctggtgccgtgaagctggagaaggagaagctggagcaaaacccggaggagtcccaggacatcaaagctctgcagaaagaactcgagcaatttgccaagctcctgaagcagaagaggatcaccctgggatatacacaggccgatgtggggctcaccctgggggttctatttgggaaggtattcagccaaacgaccatctgccgctttgaggctctgcagcttagcttcaagaacatgtgtaagctgcggcccttgctgcagaagtgggtggaggaagctgacaacaatgaaaatcttcaggagatatgcaaagcagaaaccctcgtgcaggcccgaaagagaaagcgaaccagtatcgagaaccgagtgagaggcaacctggagaatttgttcctgcagtgcccgaaacccacactgcagcagatcagccacatcgcccagcagcttgggctcgagaaggatgtggtccgagtgtggttctgtaaccggcgccagaagggcaagcgatcaagcagcgactatgcacaacgagaggattttgaggctgctgggtctcctttctcagggggaccagtgtcctttcctctggccccagggccccattttggtaccccaggctatgggagccctcacttcactgcactgtactcctcggtccctttccctgagggggaagcctttccccctgtctccgtcaccactctgggctctcccatgcattcaaactga

SEQ ID NO: 3 - DNA, 954 bp, Sox2
atgtacaacatgatggagacggagctgaagccgccgggcccgcagcaaacttcggggggcggcggcggcaactccaccgcggcggcggccggcggcaaccagaaaaacagcccggaccgcgtcaagcggcccatgaatgccttcatggtgtggtcccgcgggcagcggcgcaagatggcccaggagaaccccaagatgcacaactcggagatcagcaagcgcctgggcgccgagtggaaacttttgtcggagacggagaagcggccgttcatcgacgaggctaagcggctgcgagcgctgcacatgaaggagcacccggattataaataccggccccggcggaaaaccaagacgctcatgaagaaggataagtacacgctgcccggcgggctgctggcccccggcggcaatagcatggcgagcggggtcggggtgggcgccggcctgggcgcgggcgtgaaccagcgcatggacagttacgcgcacatgaacggctggagcaacggcagctacagcatgatgcaggaccagctgggctacccgcagcacccgggcctcaatgcgcacggcgcagcgcagatgcagcccatgcaccgctacgacgtgagcgccctgcagtacaactccatgaccagctcgcagacctacatgaacggctcgcccacctacagcatgtcctactcgcagcagggcacccctggcatggctcttggctccatgggttcggtggtcaagtccgaggccagctccagcccccctgtggttacctcttcctcccactccagggcgccctgccaggccggggacctccgggacatgatcagcatgtatctccccggcgccgaggtgccggaacccgccgcccccagcagacttcacatgtcccagcactaccagagcggcccggtgcccggcacggccattaacggcacactgcccctctcacacatgtga

SEQ ID NO: 4 - DNA, 630 bp, Lin28
atgggctccgtgtccaaccagcagtttgcaggtggctgcgccaaggcggcagaagaggcgcccgaggaggcgccggaggacgcggcccgggcggcggacgagcctcagctgctgcacggtgcgggcatctgtaagtggttcaacgtgcgcatggggttcggcttcctgtccatgaccgcccgcgccggggtcgcgctcgaccccccagtggatgtctttgtgcaccagagtaagctgcacatggaagggttccggagcttgaaggagggtgaggcagtggagttcacctttaagaagtcagccaagggtctggaatccatccgtgtcaccggacctggtggagtattctgtattgggagtgagaggcggccaaaaggaaagagcatgcagaagcgcagatcaaaaggagacaggtgctacaactgtggaggtctagatcatcatgccaaggaatgcaagctgccaccccagcccaagaagtgccacttctgccagagcatcagccatatggtagcctcatgtccgctgaaggcccagcagggccctagtgcacagggaaagccaacctactttcgagaggaagaagaagaaatccacagccctaccctgctcccggaggcacagaattga

SEQ ID NO: 5 - DNA, 918 bp, Nanog
atgagtgtggatccagcttgtccccaaagcttgccttgctttgaagcatccgactgtaaagaatcttcacctatgcctgtgatttgtgggcctgaagaaaactatccatccttgcaaatgtcttctgctgagatgcctcacacggagactgtctctcctcttccctcctccatggatctgcttattcaggacagccctgattcttccaccagtcccaaaggcaaacaacccacttctgcagagaatagtgtcgcaaaaaaggaagacaaggtcccagtcaagaaacagaagaccagaactgtgttctcttccacccagctgtgtgtactcaatgatagatttcagagacagaaatacctcagcctccagcagatgcaagaactctccaacatcctgaacctcagctacaaacaggtgaagacctggttccagaaccagagaatgaaatctaagaggtggcagaaaaacaactggccgaagaatagcaatggtgtgacgcagaaggcctcagcacctacctaccccagcctctactcttcctaccaccagggatgcctggtgaacccgactgggaaccttccaatgtggagcaaccagacctggaacaattcaacctggagcaaccagacccagaacatccagtcctggagcaaccactcctggaacactcagacctggtgcacccaatcctggaacaatcaggcctggaacagtcccttctataactgtggagaggaatctctgcagtcctgcatgcagttccagccaaattctcctgccagtgacttggaggctgctttggaagctgctggggaaggccttaatgtaatacagcagaccactaggtattttagtactccacaaaccatggatttattcctaaactactccatgaacatgcaacctgaagacgtgtga

SEQ ID NO: 6 - DNA, 8060 bp, Lentivirus harboring Stella
  misc_feature (3604)..(4083): Sequence for Stella
cggaccgccactgccaattacctgtggtttcatttactctaaacctgtgattcctctgaattattttcattttaaagaaattgtatttgttaaatatgtactacaaacttagtagttggaagggctaattcactcccaaagaagacaagatatccttgatctgtggatctaccacacacaaggctacttccctgattagcagaactacacaccagggccaggggtcagatatccactgacctttggatggtgctacaagctagtaccagttgagccagataaggtagaagaggccaataaaggagagaacaccagcttgttacaccctgtgagcctgcatgggatggatgacccggagagagaagtgttagagtggaggtttgacagccgcctagcatttcatcacgtggcccgagagctgcatccggagtacttcaagaactgctgatatcgagcttgctacaagggactttccgctggggactttccagggaggcgtggcctgggcgggactggggagtggcgagccctcagatcctgcatataagcagctgctttttgcctgtactgggtctctctggttagaccagatctgagcctgggagctctctggctaactagggaacccactgcttaagcctcaataaagcttgccttgagtgcttcaagtagtgtgtgcccgtctgttgtgtgactctggtaactagagatccctcagacccttttagtcagtgtggaaaatctctagcagtggcgcccgaacagggacttgaaagcgaaagggaaaccagaggagctctctcgacgcaggactcggcttgctgaagcgcgcacggcaagaggcgaggggcggcgactggtgagtacgccaaaaattttgactagcggaggctagaaggagagagatgggtgcgagagcgtcagtattaagcgggggagaattagatcgcgatgggaaaaaattcggttaaggccagggggaaagaaaaaatataaattaaaacatatagtatgggcaagcagggagctagaacgattcgcagttaatcctggcctgttagaaacatcagaaggctgtagacaaatactgggacagctacaaccatcccttcagacaggatcagaagaacttagatcattatataatacagtagcaaccctctattgtgtgcatcaaaggatagagataaaagacaccaaggaagctttagacaagatagaggaagagcaaaacaaaagtaagaccaccgcacagcaagcggccgctgatcttcagacctggaggaggagatatgagggacaattggagaagtgaattatataaatataaagtagtaaaaattgaaccattaggagtagcacccaccaaggcaaagagaagagtggtgcagagagaaaaaagagcagtgggaataggagctttgttccttgggttcttgggagcagcaggaagcactatgggcgcagcgtcaatgacgctgacggtacaggccagacaattattgtctggtatagtgcagcagcagaacaatttgctgagggctattgaggcgcaacagcatctgttgcaactcacagtctggggcatcaagcagctccaggcaagaatcctggctgtggaaagatacctaaaggatcaacagctcctggggatttggggttgctctggaaaactcatttgcaccactgctgtgccttggaatgctagttggagtaataaatctctggaacagatttggaatcacacgacctggatggagtgggacagagaaattaacaattacacaagcttaatacactccttaattgaagaatcgcaaaaccagcaagaaaagaatgaacaagaattattggaattagataaatgggcaagtttgtggaattggtttaacataacaaattggctgtggtatataaaattattcataatgatagtaggaggcttggtaggtttaagaatagtttttgctgtactttctatagtgaatagagttaggcagggatattcaccattatcgtttcagacccacctcccaaccccgaggggacccgacaggcccgaaggaatagaagaagaaggtggagagagagacagagacagatccattcgattagtgaacggatctcgacggtatcgccacaaatggcagtattcatccacaattttaaaagaaagggggggattggggggtacagtgcaggggaaagaatagtagacataatagcaacagacatacaaactaaagaattacaaaaacaaattacaaaaattcaaaattttcgggtttattacagggacagcagagatccactttggtcgataagctttgcaaagatggataaagttttaaacagagaggaatctttgcagctaatggaccttctaggtcttgaaaggagtgggaattggctccggtgcccgtcagtgggcagagcgcacatcgcccacagtccccgagaagttggggggaggggtcggcaattgaaccggtgcctagagaaggtggcgcggggtaaactgggaaagtgatgtcgtgtactggctccgcctttttcccgagggtgggggagaaccgtatataagtgcagtagtcgccgtgaacgttctttttcgcaacgggtttgccgccagaacacaggtaagtgccgtgtgtggttcccgcgggcctggcctctttacgggttatggcccttgcgtgccttgaattacttccacctggctgcagtacgtgattcttgatcccgagcttcgggttggaagtgggtgggagagttcgaggccttgcgcttaaggagccccttcgcctcgtgcttgagttgaggcctggcctgggcgctggggccgccgcgtgcgaatctggtggcaccttcgcgcctgtctcgctgctttcgataagtctctagccatttaaaatttttgatgacctgctgcgacgctttttttctggcaagatagtcttgtaaatgcgggccaagatctgcacactggtatttcggtttttggggccgcgggcggcgacggggcccgtgcgtcccagcgcacatgttcggcgaggcggggcctgcgagcgcggccaccgagaatcggacgggggtagtctcaagctggccggcctgctctggtgcctggcctcgcgccgccgtgtatcgccccgccctgggcggcaaggctggcccggtcggcaccagttgcgtgagcggaaagatggccgcttcccggccctgctgcagggagctcaaaatggaggacgcggcgctcgggagagcgggcgggtgagtcacccacacaaaggaaaagggcctttccgtcctcagccgtcgcttcatgtgactccacggagtaccgggcgccgtccaggcacctcgattagttctcgagcttttggagtacgtcgtctttaggttggggggaggggttttatgcgatggagtttccccacactgagtgggtggagactgaagttaggccagcttggcacttgatgtaattctccttggaatttgccctttttgagtttggatcttggttcattctcaagcctcagacagtggttcaaagtttttttcttccatttcaggtgtcgtgaggaattcgcgatcgccatggacccatcacagtttaatccaacctacatcccagggtctccacaaatgctcaccgaagaaaattcccgggacgattcaggggcctctcaaatctcctccgagacgttgataaagaaccttagtaacttgactatcaacgctagtagcgaatctgtttcccctctatcggaagctttactccgtcgagagtctgtaggagcagcagtcctcagggaaatcgaagatgagtggctttacagcaggagaggagtaagaacattgctgtctgtgcagagagaaaagatggcaagattgagatacatgttactcggcggagttcgtacgcatgaaagaagaccaacaaacaaggagcctaagggagttaagaaggaatcaagaccattcaaatgtccctgcagtttctgcgtgtctaatggatgggatccttctgagaatgctagaatagggaatcaagacaccaagccacttcagccataataggtttaaacatcgatggcctcgagaaagcggccgcccccacgcgtaaactagttcgaaggatccgcatgcatctagggcggccaattccgcccctctccctcccccccccctaacgttactggccgaagccgcttggaataaggccggtgtgcgtttgtctatatgtgattttccaccatattgccgtcttttggcaatgtgagggcccggaaacctggccctgtcttcttgacgagcattcctaggggtctttcccctctcgccaaaggaatgcaaggtctgttgaatgtcgtgaaggaagcagttcctctggaagcttcttgaagacaaacaacgtctgtagcgaccctttgcaggcagcggaaccccccacctggcgacaggtgcctctgcggccaaaagccacgtgtataagatacacctgcaaaggcggcacaaccccagtgccacgttgtgagttggatagttgtggaaagagtcaaatggctctcctcaagcgtattcaacaaggggctgaaggatgcccagaaggtaccccattgtatgggatctgatctggggcctcggtgcacatgctttacatgtgtttagtcgaggttaaaaaaacgtctaggccccccgaaccacggggacgtggttttcctttgaaaaacacgatgataagcttgccacaacccacaaggagacgaccttccatgaccgagtacaagcccacggtgcgcctcgccacccgcgacgacgtcccccgggccgtacgcaccctcgccgccgcgttcgccgactaccccgccacgcgccacaccgtcgacccggaccgccacatcgagcgggtcaccgagctgcaagaactcttcctcacgcgcgtcgggctcgacatcggcaaggtgtgggtcgcggacgacggcgccgcggtggcggtctggaccacgccggagagcgtcgaagcgggggcggtgttcgccgagatcggcccgcgcatggccgagttgagcggttcccggctggccgcgcagcaacagatggaaggcctcctggcgccgcaccggcccaaggagcccgcgtggttcctggccaccgtcggcgtctcgcccgaccaccagggcaagggtctgggcagcgccgtcgtgctccccggagtggaggcggccgagcgcgccggggtgcccgccttcctggagacctccgcgccccgcaacctccccttctacgagcggctcggcttcaccgtcaccgccgacgtcgagtgcccgaaggaccgcgcgacctggtgcatgacccgcaagcccggtgcctgataataggcggccgctcgagacctagaaaaacatggagcaatcacaagtagcaatacagcagctaccaatgctgattgtgcctggctagaagcacaagaggaggaggaggtgggttttccagtcacacctcaggtacctttaagaccaatgacttacaaggcagctgtagatcttagccactttttaaaagaaaaggggggactggaagggctaattcactcccaacgaagacaagatctgctttttgcttgtactgggtctctctggttagaccagatctgagcctgggagctctctggctaactagggaacccactgcttaagcctcaataaagcttgccttgagtgcttcaagtagtgtgtgcccgtctgttgtgtgactctggtaactagagatccctcagacccttttagtcagtgtggaaaatctctagcagtagtagttcatgtcatcttattattcagtatttataacttgcaaagaaatgaatatcagagagtgagaggccttgacattataatagatttagcaggaattgaactaggagtggagcacacaggcaaagttctagagctcgctgatcagcctcgactgtgccttctagttgccagccatctgttgtttgcccctcccccgtgccttccttgaccctggaaggtgccactcccactgtcctttcctaataaaatgaggaaattgcatcgcattgtctgagtaggtgtcattctattctggggggtggggtggggcaggacagcaagggggaggattgggaagacaatagcaggcatgctggggatgcggtgggctctatggcttctgaggcggaaagaaccagctgggggcgcgcccctcgaggccgccatggtcatagctgtttgacgtcaggtggcacttttcggggaaatgtgcgcggaacccctatttgtttatttttctaaatacattcaaatatgtatccgctcatgagacaataaccctgataaatgcttcaataatattgaaaaaggaagagtatgagtattcaacatttccgtgtcgcccttattcccttttttgcggcattttgccttcctgtttttgctcacccagaaacgctggtgaaagtaaaagatgctgaagatcagttgggtgcacgagtgggttacatcgaactggatctcaacagcggtaagatccttgagagttttcgccccgaagaacgttttccaatgatgagcacttttaaagttctgctatgtggcgcggtattatcccgtattgacgccgggcaagagcaactcggtcgccgcatacactattctcagaatgacttggttgagtactcaccagtcacagaaaagcatcttacggatggcatgacagtaagagaattatgcagtgctgccataaccatgagtgataacactgcggccaacttacttctgacaacgatcggaggaccgaaggagctaaccgcttttttgcacaacatgggggatcatgtaactcgccttgatcgttgggaaccggagctgaatgaagccataccaaacgacgagcgtgacaccacgatgcctgtagcaatggcaacaacgttgcgcaaactattaactggcgaactacttactctagcttcccggcaacaattaatagactggatggaggcggataaagttgcaggaccacttctgcgctcggcccttccggctggctggtttattgctgataaatctggagccggtgagcgtgggtctcgcggtatcattgcagcactggggccagatggtaagccctcccgtatcgtagttatctacacgacggggagtcaggcaactatggatgaacgaaatagacagatcgctgagataggtgcctcactgattaagcattggtaactgtcagaccaagtttactcatatatactttagattgatttaaaacttcatttttaatttaaaaggatctaggtgaagatcctttttgataatctcatgaccaaaatcccttaacgtgagttttcgttccactgagcgtcagaccccgtagaaaagatcaaaggatcttcttgagatcctttttttctgcgcgtaatctgctgcttgcaaacaaaaaaaccaccgctaccagcggtggtttgtttgccggatcaagagctaccaactctttttccgaaggtaactggcttcagcagagcgcagataccaaatactgtccttctagtgtagccgtagttaggccaccacttcaagaactctgtagcaccgcctacatacctcgctctgctaatcctgttaccagtggctgctgccagtggcgataagtcgtgtcttaccgggttggactcaagacgatagttaccggataaggcgcagcggtcgggctgaacggggggttcgtgcacacagcccagcttggagcgaacgacctacaccgaactgagatacctacagcgtgagcattgagaaagcgccacgcttcccgaagggagaaaggcggacaggtatccggtaagcggcagggtcggaacaggagagcgcacgagggagcttccagggggaaacgcctggtatctttatagtcctgtcgggtttcgccacctctgacttgagcgtcgatttttgtgatgctcgtcaggggggcggagcctatggaaaaacgccagcaacgcggcctttttacggttcctggccttttgc

SEQ ID NO: 7 - DNA, 19 bp, Artificial
  Synthetic oligonucleotide
cagtgcccgaaacccacac

SEQ ID NO: 8 - DNA, 24 bp, Artificial
  Synthetic oligonucleotide
agaggaactgcttccttcacgaca

SEQ ID NO: 9 - DNA, 20 bp, Artificial
  Synthetic oligonucleotide
cagaaggcctcagcacctac

SEQ ID NO: 10 - DNA, 20 bp, Artificial
  Synthetic oligonucleotide
tacctcttcctcccactcca

SEQ ID NO: 11 - DNA, 20 bp, Artificial
  Synthetic oligonucleotide
aagcgcagatcaaaaggaga

SEQ ID NO: 12 - DNA, 20 bp, Artificial
  Synthetic oligonucleotide
agtttgtgccagggtttttg

SEQ ID NO: 13 - DNA, 20 bp, Artificial
  Synthetic oligonucleotide
acttcaccttccctccaacc